European Patent Application EP 4 803 530 A1, published September 9, 2026. Title: 核苷及核苷酸类似物、含核苷酸类似物的双链寡核苷酸与缀合物及其应用. Applicant: 北京炫景瑞医药科技有限公司. The sequence listing filed with the application follows.

SEQUENCE LISTING (12 sequences)

SEQ ID NO: 1 - RNA, 19 nt, artificial sequence
  source 1..19: mol_type = genomic RNA
cagacagacaagaccatct

SEQ ID NO: 2 - RNA, 19 nt, artificial sequence
  source 1..19: mol_type = genomic RNA
ccaagagcaccaagaacta

SEQ ID NO: 3 - RNA, 19 nt, artificial sequence
  source 1..19: mol_type = genomic RNA
atgtgaaagtcatcgacaa

SEQ ID NO: 4 - RNA, 21 nt, artificial sequence
  source 1..21: mol_type = genomic RNA
agatggtcttgtctgtctgtt

SEQ ID NO: 5 - RNA, 21 nt, artificial sequence
  source 1..21: mol_type = genomic RNA
tagttcttggtgctcttggtt

SEQ ID NO: 6 - RNA, 21 nt, artificial sequence
  source 1..21: mol_type = genomic RNA
ttgtcgatgactttcacattc

SEQ ID NO: 7 - DNA, 20 bp, artificial sequence
  source 1..20: mol_type = genomic DNA
ccagctccccattagctctg

SEQ ID NO: 8 - DNA, 22 bp, artificial sequence
  source 1..22: mol_type = genomic DNA
gcacttgcctctttaggaagtc

SEQ ID NO: 9 - DNA, 19 bp, artificial sequence
  source 1..19: mol_type = genomic DNA
tgcaccaccaactgcttag

SEQ ID NO: 10 - DNA, 19 bp, artificial sequence
  source 1..19: mol_type = genomic DNA
ggatgcagggatgatgttc

SEQ ID NO: 11 - DNA, 23 bp, artificial sequence
  source 1..23: mol_type = genomic DNA
gaggagcagctaaccaacttaat

SEQ ID NO: 12 - DNA, 23 bp, artificial sequence
  source 1..23: mol_type = genomic DNA
tctgcatgtgctgttgacttaat